European Patent Application EP 4 154 890 A1, published March 29, 2023. Title: PHARMACEUTICAL COMPOSITION FOR PREVENTING OR TREATING PANCREATIC CANCER ASSOCIATED WITH RON MUTATION AND METHOD USING THE SAME. Applicant: Wellmarker Bio Co., LTD. The sequence listing filed with the application follows.

SEQUENCE LISTING (8 sequences)

SEQ ID NO: 1 - protein, 188 aa, Homo sapiens [sequence omitted]

SEQ ID NO: 2 - DNA, 3732 bp, Artificial Sequence
  RON 155 cDNA
atggagctcctcccgccgctgcctcagtccttcctgttgctgctgctgttgcctgccaagcccgcggcgggcgaggactggcagtgcccgcgcaccccctacgcggcctctcgcgactttgacgtgaagtacgtggtgcccagcttctccgccggaggcctggtacaggccatggtgacctacgagggcgacagaaatgagagtgctgtgtttgtagccatacgcaatcgcctgcatgtgcttgggcctgacctgaagtctgtccagagcctggccacgggccctgctggagaccctggctgccagacgtgtgcagcctgtggcccaggaccccacggccctcccggtgacacagacacaaaggtgctggtgctggatcccgcgctgcctgcgctggtcagttgtggctccagcctgcagggccgctgcttcctgcatgacctagagccccaagggacagccgtgcatctggcagcgccagcctgcctcttctcagcccaccataaccggcccgatgactgccccgactgtgtggccagcccattgggcacccgtgtaactgtggttgagcaaggccaggcctcctatttctacgtggcatcctcactggacgcagccgtggctgccagcttcagcccacgctcagtgtctatcaggcgtctcaaggctgacgcctcgggattcgcaccgggctttgtggcgttgtcagtgctgcccaagcatcttgtctcctacagtattgaatacgtgcacagcttccacacgggagccttcgtgtacttcctgactgtacagccggccagcgtgacagatgatcctagtgccctgcacacacgcctggcacggcttagcgccactgagccagagttgggtgactatcgggagctggtcctcgactgcagatttgctccaaaacgcaggcgccggggggccccagaaggcggacagccctaccctgtgctgcgggtggcccactccgctccagtgggtgcccaacttgccactgagctgagcatcgccgagggccaggaagtactatttggggtctttgtgactggcaaggatggtggtcctggcgtgggccccaactctgtcgtctgtgccttccccattgacctgctggacacactaattgatgagggtgtggagcgctgttgtgaatccccagtccatccaggcctccggcgaggcctcgacttcttccagtcgcccagtttttgccccaacccgcctggcctggaagccctcagccccaacaccagctgccgccacttccctctgctggtcagtagcagcttctcacgtgtggacctattcaatgggctgttgggaccagtacaggtcactgcattgtatgtgacacgccttgacaacgtcacagtggcacacatgggcacaatggatgggcgtatcctgcaggtggagctggtcaggtcactaaactacttgctgtatgtgtccaacttctcactgggtgacagtgggcagcccgtgcagcgggatgtcagtcgtcttggggaccacctactctttgcctctggggaccaggttttccaggtacctatccaaggccctggctgccgccacttcctgacctgtgggcgttgcctaagggcatggcatttcatgggctgtggctggtgtgggaacatgtgcggccagcagaaggagtgtcctggctcctggcaacaggaccactgcccacctaagcttactgaggagccagtgctgatagcagtgcaacccctctttggcccacgggcaggaggcacctgtctcactcttgaaggccagagtctgtctgtaggcaccagccgggctgtgctggtcaatgggactgagtgtctgctagcacgggtcagtgaggggcagcttttatgtgccacaccccctggggccacggtggccagtgtcccccttagcctgcaggtggggggtgcccaggtacctggttcctggaccttccagtacagagaagaccctgtcgtgctaagcatcagccccaactgtggctacatcaactcccacatcaccatctgtggccagcatctaacttcagcatggcacttagtgctgtcattccatgacgggcttagggcagtggaaagcaggcagtgtgagaggcagcttccagagcagcagctgtgccgccttcctgaatatgtggtccgagacccccagggatgggtggcagggaatctgagtgcccgaggggatggagctgctggctttacactgcctggctttcgcttcctacccccaccccatccacccagtgccaacctagttccactgaagcctgaggagcatgccattaagtttgaggtctgcgtagatggtgaatgtcatatcctgggtagagtggtgcggccagggccagatggggtcccacagagcacgctccttggtatcctgctgcctttgctgctgcttgtggctgcactggcgactgcactggtcttcagctactggtggcggaggaagcagctagttcttcctcccaacctgaatgacctggcatccctggaccagactgctggagccacacccctgcctattctgtactcgggctctgactacagaagtggccttgcactccctgccattgatggtctggattccaccacttgtgtccatggagcatccttctccgatagtgaagatgaatcctgtgtgccactgctgcggaaagagtccatccagctaagggacctggactctgcgctcttggctgaggtcaaggatgtgctgattccccatgagcgggtggtcacccacagtgaccgagtcattggcaaaggccactttggagttgtctaccacggagaatacatagaccaggcccagaatcgaatccaatgtgccatcaagtcactaagtcgcatcacagagatgcagcaggtggaggccttcctgcgagaggggctgctcatgcgtggcctgaaccacccgaatgtgctggctctcattggtatcatgttgccacctgagggcctgccccatgtgctgctgccctatatgtgccacggtgacctgctccagttcatccgctcacctcagcggaaccccaccgtgaaggacctcatcagctttggcctgcaggtagcccgcggcatggagtacctggcagagcagaagtttgtgcacagggacctggctgcgcggaactgcatgctggacgagtcattcacagtcaaggtggctgactttggtttggcccgcgacatcctggacagggagtactatagtgttcaacagcatcgccacgctcgcctacctgtgaagtggatggcgctggagagcctgcagacctatagatttaccaccaagtctgatgtgtggtcatttggtgtgctgctgtgggaactgctgacacggggtgccccaccataccgccacattgacccttttgaccttacccacttcctggcccagggtcggcgcctgccccagcctgagtattgccctgattctctgtaccaagtgatgcagcaatgctgggaggcagacccagcagtgcgacccaccttcagagtactagtgggggaggtggagcagatagtgtctgcactgcttggggaccattatgtgcagctgccagcaacctacatgaacttgggccccagcacctcgcatgagatgaatgtgcgtccagaacagccgcagttctcacccatgccagggaatgtacgccggccccggccactctcagagcctcctcggcccacttga

SEQ ID NO: 3 - DNA, 3879 bp, Artificial Sequence
  RON 160 cDNA
atggagctcctcccgccgctgcctcagtccttcctgttgctgctgctgttgcctgccaagcccgcggcgggcgaggactggcagtgcccgcgcaccccctacgcggcctctcgcgactttgacgtgaagtacgtggtgcccagcttctccgccggaggcctggtacaggccatggtgacctacgagggcgacagaaatgagagtgctgtgtttgtagccatacgcaatcgcctgcatgtgcttgggcctgacctgaagtctgtccagagcctggccacgggccctgctggagaccctggctgccagacgtgtgcagcctgtggcccaggaccccacggccctcccggtgacacagacacaaaggtgctggtgctggatcccgcgctgcctgcgctggtcagttgtggctccagcctgcagggccgctgcttcctgcatgacctagagccccaagggacagccgtgcatctggcagcgccagcctgcctcttctcagcccaccataaccggcccgatgactgccccgactgtgtggccagcccattgggcacccgtgtaactgtggttgagcaaggccaggcctcctatttctacgtggcatcctcactggacgcagccgtggctgccagcttcagcccacgctcagtgtctatcaggcgtctcaaggctgacgcctcgggattcgcaccgggctttgtggcgttgtcagtgctgcccaagcatcttgtctcctacagtattgaatacgtgcacagcttccacacgggagccttcgtgtacttcctgactgtacagccggccagcgtgacagatgatcctagtgccctgcacacacgcctggcacggcttagcgccactgagccagagttgggtgactatcgggagctggtcctcgactgcagatttgctccaaaacgcaggcgccggggggccccagaaggcggacagccctaccctgtgctgcgggtggcccactccgctccagtgggtgcccaacttgccactgagctgagcatcgccgagggccaggaagtactatttggggtctttgtgactggcaaggatggtggtcctggcgtgggccccaactctgtcgtctgtgccttccccattgacctgctggacacactaattgatgagggtgtggagcgctgttgtgaatccccagtccatccaggcctccggcgaggcctcgacttcttccagtcgcccagtttttgccccaacccgcctggcctggaagccctcagccccaacaccagctgccgccacttccctctgctggtcagtagcagcttctcacgtgtggacctattcaatgggctgttgggaccagtacaggtcactgcattgtatgtgacacgccttgacaacgtcacagtggcacacatgggcacaatggatgggcgtatcctgcaggtggagctggtcaggtcactaaactacttgctgtatgtgtccaacttctcactgggtgacagtgggcagcccgtgcagcgggatgtcagtcgtcttggggaccacctactctttgcctctggggaccaggttttccaggtacctatccaaggccctggctgccgccacttcctgacctgtgggcgttgcctaagggcatggcatttcatgggctgtggctggtgtgggaacatgtgcggccagcagaaggagtgtcctggctcctggcaacaggaccactgcccacctaagcttactgaggagccagtgctgatagcagtgcaacccctctttggcccacgggcaggaggcacctgtctcactcttgaaggccagagtctgtctgtaggcaccagccgggctgtgctggtcaatgggactgagtgtctgctagcacgggtcagtgaggggcagcttttatgtgccacaccccctggggccacggtggccagtgtcccccttagcctgcaggtggggggtgcccaggtacctggttcctggaccttccagtacagagaagaccctgtcgtgctaagcatcagccccaactgtggctacatcaactcccacatcaccatctgtggccagcatctaacttcagcatggcacttagtgctgtcattccatgacgggcttagggcagtggaaagcaggcagtgtgagaggcagcttccagagcagcagctgtgccgccttcctgaatatgtggtccgagacccccagggatgggtggcagggaatctgagtgcccgaggggatggagctgctggctttacactgcctggctttcgcttcctacccccaccccatccacccagtgccaacctagttccactgaagcctgaggagcatgccattaagtttgagtatattgggctgggcgctgtggctgactgtgtgggtatcaacgtgaccgtgggtggtgagagctgccagcacgagttccggggggacatggttgtctgccccctgcccccatccctgcagcttggccaggatggtgccccattgcaggtctgcgtagatggtgaatgtcatatcctgggtagagtggtgcggccagggccagatggggtcccacagagcacgctccttggtatcctgctgcctttgctgctgcttgtggctgcactggcgactgcactggtcttcagctactggtggcggaggaagcagctagttcttcctcccaacctgaatgacctggcatccctggaccagactgctggagccacacccctgcctattctgtactcgggctctgactacagaagtggccttgcactccctgccattgatggtctggattccaccacttgtgtccatggagcatccttctccgatagtgaagatgaatcctgtgtgccactgctgcggaaagagtccatccagctaagggacctggactctgcgctcttggctgaggtcaaggatgtgctgattccccatgagcgggtggtcacccacagtgaccgagtcattggcaaaggccactttggagttgtctaccacggagaatacatagaccaggcccagaatcgaatccaatgtgccatcaagtcactaagtcgcatcacagagatgcagcaggtggaggccttcctgcgagaggggctgctcatgcgtggcctgaaccacccgaatgtgctggctctcattggtatcatgttgccacctgagggcctgccccatgtgctgctgccctatatgtgccacggtgacctgctccagttcatccgctcacctcagcggaaccccaccgtgaaggacctcatcagctttggcctgcaggtagcccgcggcatggagtacctggcagagcagaagtttgtgcacagggacctggctgcgcggaactgcatgctggacgagtcattcacagtcaaggtggctgactttggtttggcccgcgacatcctggacagggagtactatagtgttcaacagcatcgccacgctcgcctacctgtgaagtggatggcgctggagagcctgcagacctatagatttaccaccaagtctgatgtgtggtcatttggtgtgctgctgtgggaactgctgacacggggtgccccaccataccgccacattgacccttttgaccttacccacttcctggcccagggtcggcgcctgccccagcctgagtattgccctgattctctgtaccaagtgatgcagcaatgctgggaggcagacccagcagtgcgacccaccttcagagtactagtgggggaggtggagcagatagtgtctgcactgcttggggaccattatgtgcagctgccagcaacctacatgaacttgggccccagcacctcgcatgagatgaatgtgcgtccagaacagccgcagttctcacccatgccagggaatgtacgccggccccggccactctcagagcctcctcggcccacttga

SEQ ID NO: 4 - DNA, 4056 bp, Artificial Sequence
  RON 165 cDNA
atggagctcctcccgccgctgcctcagtccttcctgttgctgctgctgttgcctgccaagcccgcggcgggcgaggactggcagtgcccgcgcaccccctacgcggcctctcgcgactttgacgtgaagtacgtggtgcccagcttctccgccggaggcctggtacaggccatggtgacctacgagggcgacagaaatgagagtgctgtgtttgtagccatacgcaatcgcctgcatgtgcttgggcctgacctgaagtctgtccagagcctggccacgggccctgctggagaccctggctgccagacgtgtgcagcctgtggcccaggaccccacggccctcccggtgacacagacacaaaggtgctggtgctggatcccgcgctgcctgcgctggtcagttgtggctccagcctgcagggccgctgcttcctgcatgacctagagccccaagggacagccgtgcatctggcagcgccagcctgcctcttctcagcccaccataaccggcccgatgactgccccgactgtgtggccagcccattgggcacccgtgtaactgtggttgagcaaggccaggcctcctatttctacgtggcatcctcactggacgcagccgtggctgccagcttcagcccacgctcagtgtctatcaggcgtctcaaggctgacgcctcgggattcgcaccgggctttgtggcgttgtcagtgctgcccaagcatcttgtctcctacagtattgaatacgtgcacagcttccacacgggagccttcgtatacttcctgactgtacagccggccagcgtgacagatgatcctagtgccctgcacacacgcctggcacggcttagcgccactgagccagagttgggtgactatcgggagctggtcctcgactgcagatttgctccaaaacgcaggcgccggggggccccagaaggcggacagccctaccctgtgctgcgggtggcccactccgctccagtgggtgcccaacttgccactgagctgagcatcgccgagggccaggaagtactatttggggtctttgtgactggcaaggatggtggtcctggcgtgggccccaactctgtcgtctgtgccttccccattgacctgctggacacactaattgatgagggtgtggagcgctgttgtgaatccccagtccatccaggcctccggcgaggcctcgacttcttccagtcgcccagtttttgccccaacccgcctggcctggaagccctcagccccaacaccagctgccgccacttccctctgctggtcagtagcagcttctcacgtgtggacctattcaatgggctgttgggaccagtacaggtcactgcattgtatgtgacacgccttgacaacgtcacagtggcacacatgggcacaatggatgggcgtatcctgcaggtggagctggtcaggtcactaaactacttgctgtatgtgtccaacttctcactgggtgacagtgggcagcccgtgcagcgggatgtcagtcgtcttggggaccacctactctttgcctctggggaccaggttttccaggtacctatccaaggccctggctgccgccacttcctgacctgtgggcgttgcctaagggcatggcatttcatgggctgtggctggtgtgggaacatgtgcggccagcagaaggagtgtcctggctcctggcaacaggaccactgcccacctaagcttactgagttccacccccacagtggacctctaaggggcagtacaaggctgaccctgtgtggctccaacttctaccttcacccttctggtctggtgcctgagggaacccatcaggtcactgtgggccaaagtccctgccggccactgcccaaggacagctcaaaactcagaccagtgccccggaaagactttgtagaggagtttgagtgtgaactggagcccttgggcacccaggcagtggggcctaccaacgtcagcctcaccgtgactaacatgccaccgggcaagcacttccgggtagacggcacctccgtgctgagaggcttctctttcatggagccagtgctgatagcagtgcaacccctctttggcccacgggcaggaggcacctgtctcactcttgaaggccagagtctgtctgtaggcaccagccgggctgtgctggtcaatgggactgagtgtctgctagcacgggtcagtgaggggcagcttttatgtgccacaccccctggggccacggtggccagtgtcccccttagcctgcaggtggggggtgcccaggtacctggttcctggaccttccagtacagagaagaccctgtcgtgctaagcatcagccccaactgtggctacatcaactcccacatcaccatctgtggccagcatctaacttcagcatggcacttagtgctgtcattccatgacgggcttagggcagtggaaagcaggtgtgagaggcagcttccagagcagcagctgtgccgccttcctgaatatgtggtccgagacccccagggatgggtggcagggaatctgagtgcccgaggggatggagctgctggctttacactgcctggctttcgcttcctacccccaccccatccacccagtgccaacctagttccactgaagcctgaggagcatgccattaagtttgaggtctgcgtagatggtgaatgtcatatcctgggtagagtggtgcggccagggccagatggggtcccacagagcacgctccttggtatcctgctgcctttgctgctgcttgtggctgcactggcgactgcactggtcttcagctactggtggcggaggaagcagctagttcttcctcccaacctgaatgacctggcatccctggaccagactgctggagccacacccctgcctattctgtactcgggctctgactacagaagtggccttgcactccctgccattgatggtctggattccaccacttgtgtccatggagcatccttctccgatagtgaagatgaatcctgtgtgccactgctgcggaaagagtccatccagctaagggacctggactctgcgctcttggctgaggtcaaggatgtgctgattccccatgagcgggtggtcacccacagtgaccgagtcattggcaaaggccactttggagttgtctaccacggagaatacatagaccaggcccagaatcgaatccaatgtgccatcaagtcactaagtcgcatcacagagatgcagcaggtggaggccttcctgcgagaggggctgctcatgcgtggcctgaaccacccgaatgtgctggctctcattggtatcatgttgccacctgagggcctgccccatgtgctgctgccctatatgtgccacggtgacctgctccagttcatccgctcacctcagcggaaccccaccgtgaaggacctcatcagctttggcctgcaggtagcccgcggcatggagtacctggcagagcagaagtttgtgcacagggacctggctgcgcggaactgcatgctggacgagtcattcacagtcaaggtggctgactttggtttggcccgcgacatcctggacagggagtactatagtgttcaacagcatcgccacgctcgcctacctgtgaagtggatggcgctggagagcctgcagacctatagatttaccaccaagtctgatgtgtggtcatttggtgtgctgctgtgggaactgctgacacggggtgccccaccataccgccacattgacccttttgaccttacccacttcctggcccagggtcggcgcctgccccagcctgagtattgccctgattctctgtaccaagtgatgcagcaatgctgggaggcagacccagcagtgcgacccaccttcagagtactagtgggggaggtggagcagatagtgtctgcactgcttggggaccattatgtgcagctgccagcaacctacatgaacttgggccccagcacctcgcatgagatgaatgtgcgtccagaacagccgcagttctcacccatgccagggaatgtacgccggccccggccactctcagagcctcctcggcccacttga

SEQ ID NO: 5 - DNA, 21 bp, Artificial Sequence
  RON d5_6 sense primer
gagctggtcaggtcactaaac

SEQ ID NO: 6 - DNA, 21 bp, Artificial Sequence
  RON d5_6 antisense primer
cagacactcagtcccattgac

SEQ ID NO: 7 - DNA, 20 bp, Artificial Sequence
  RON d11 sense primer
atctgtggccagcatctaac

SEQ ID NO: 8 - DNA, 20 bp, Artificial Sequence
  RON d11 antisense primer
aaaggcagcaggataccaag